European Patent Specification EP 3 954 767 B1, published June 17, 2026. Title: A modified polypeptide of glutamine synthetase and a method for L-glutamine using the same. Applicant: CJ CheilJedang Corporation. The sequence listing filed with the application follows.

SEQUENCE LISTING (29 sequences)

SEQ ID NO: 1 - protein, 477 aa, Artificial Sequence
  Corynebacterium glutamicum ATCC13032 Glutamine synthetase a.a.
VAFETPEEIVKFIKDENVEFVDVRFTDLPGTEQHFSIPAASFDADTIEEGLAFDGSSIRGFTTIDESDMNLLPDLGTATLDPFRKAKTLNVKFFVHDPFTREAFSRDPRNVARKAEQYLASTGIADTCNFGAEAEFYLFDSVRYSTEMNSGFYEVDTEEGWWNRGKETNLDGTPNLGAKNRVKGGYFPVAPYDQTVDVRDDMVRNLAASGFALERFHHEVGGGQQEINYRFNTMLHAADDIQTFKYIIKNTARLHGKAATFMPKPLAGDNGSGMHAHQSLWKDGKPLFHDESGYAGLSDIARYYIGGILHHAGAVLAFTNATLNSYHRLVPGFEAPINLVYSQRNRSAAVRIPITGSNPKAKRIEFRAPDPSGNPYLGFAAMMMAGLDGIKNRIEPHAPVDKDLYELPPEEAASIPQAPTSLEASLKALQEDTDFLTESDVFTEDLIEAYIQYKYDNEISPVRLRPTPQEFELYFDC

SEQ ID NO: 2 - protein, 477 aa, Artificial Sequence
  Corynebacterium glutamicum ATCC13032 Glutamine synthetase variant a.a.
VAFETPEEIVKFIKDENVEFVDVRFTDLPGTEQHFSIPAASFDADTIEEGLAFDGSSIRGFTTIDESDMNLLPDLGTATLDPFRKAKTLNVKFFVHDPFTREAFSRDPRNVARKAEQYLASTGIADTCNFGAEAEFYLFDSVRYSTEMNSGFYEVDTEEGWWNRGKETNLDGTPNLGAKNRVKGGYFPVAPYDQTVDVRDDMVRNLAASGFALERFHHEVGGGQQEINYRFNTMLHAADDIQTFKYIIKNTARLHGKAATFMPKPLAGDNGSGMHAHQSLWKDGKPLFHDESGYAGLSDIARYYIGGILHHAGAVLAFTNATLNSYHRLVPGFEAPINLVYSQRNRSAAVRIPITGSNPKAKRIEFRAPDPSGNPYLGFAAMMMAGLDGIKNRIEPHAPVNKDLYELPPEEAASIPQAPTSLEASLKALQEDTDFLTESDVFTEDLIEAYIQYKYDNEISPVRLRPTPQEFELYFDC

SEQ ID NO: 3 - protein, 477 aa, Artificial Sequence
  Corynebacterium glutamicum ATCC13032 Glutamine synthetase variant a.a.
VAFETPEEIVKFIKDENVEFVDVRFTDLPGTEQHFSIPAASFDADTIEEGLAFDGSSIRGFTTIDESDMNLLPDLGTATLDPFRKAKTLNVKFFVHDPFTREAFSRDPRNVARKAEQYLASTGIADTCNFGAEAEFYLFDSVRYSTEMNSGFYEVDTEEGWWNRGKETNLDGTPNLGAKNRVKGGYFPVAPYDQTVDVRDDMVRNLAASGFALERFHHEVGGGQQEINYRFNTMLHAADDIQTFKYIIKNTARLHGKAATFMPKPLAGDNGSGMHAHQSLWKDGKPLFHDESGYAGLSDIARYYIGGILHHAGAVLAFTNATLNSYHRLVPGFEAPINLVYSQRNRSAAVRIPITGSNPKAKRIEFRAPDPSGNPYLGFAAMMMAGLDGIKNRIEPHAPVEKDLYELPPEEAASIPQAPTSLEASLKALQEDTDFLTESDVFTEDLIEAYIQYKYDNEISPVRLRPTPQEFELYFDC

SEQ ID NO: 4 - protein, 477 aa, Artificial Sequence
  Corynebacterium glutamicum ATCC13032 Glutamine synthetase variant a.a.
VAFETPEEIVKFIKDENVEFVDVRFTDLPGTEQHFSIPAASFDADTIEEGLAFDGSSIRGFTTIDESDMNLLPDLGTATLDPFRKAKTLNVKFFVHDPFTREAFSRDPRNVARKAEQYLASTGIADTCNFGAEAEFYLFDSVRYSTEMNSGFYEVDTEEGWWNRGKETNLDGTPNLGAKNRVKGGYFPVAPYDQTVDVRDDMVRNLAASGFALERFHHEVGGGQQEINYRFNTMLHAADDIQTFKYIIKNTARLHGKAATFMPKPLAGDNGSGMHAHQSLWKDGKPLFHDESGYAGLSDIARYYIGGILHHAGAVLAFTNATLNSYHRLVPGFEAPINLVYSQRNRSAAVRIPITGSNPKAKRIEFRAPDPSGNPYLGFAAMMMAGLDGIKNRIEPHAPVSKDLYELPPEEAASIPQAPTSLEASLKALQEDTDFLTESDVFTEDLIEAYIQYKYDNEISPVRLRPTPQEFELYFDC

SEQ ID NO: 5 - protein, 477 aa, Artificial Sequence
  Corynebacterium glutamicum ATCC13032 Glutamine synthetase variant a.a.
VAFETPEEIVKFIKDENVEFVDVRFTDLPGTEQHFSIPAASFDADTIEEGLAFDGSSIRGFTTIDESDMNLLPDLGTATLDPFRKAKTLNVKFFVHDPFTREAFSRDPRNVARKAEQYLASTGIADTCNFGAEAEFYLFDSVRYSTEMNSGFYEVDTEEGWWNRGKETNLDGTPNLGAKNRVKGGYFPVAPYDQTVDVRDDMVRNLAASGFALERFHHEVGGGQQEINYRFNTMLHAADDIQTFKYIIKNTARLHGKAATFMPKPLAGDNGSGMHAHQSLWKDGKPLFHDESGYAGLSDIARYYIGGILHHAGAVLAFTNATLNSYHRLVPGFEAPINLVYSQRNRSAAVRIPITGSNPKAKRIEFRAPDPSGNPYLGFAAMMMAGLDGIKNRIEPHAPVDHDLYELPPEEAASIPQAPTSLEASLKALQEDTDFLTESDVFTEDLIEAYIQYKYDNEISPVRLRPTPQEFELYFDC

SEQ ID NO: 6 - protein, 477 aa, Artificial Sequence
  Corynebacterium glutamicum ATCC13032 Glutamine synthetase variant a.a.
VAFETPEEIVKFIKDENVEFVDVRFTDLPGTEQHFSIPAASFDADTIEEGLAFDGSSIRGFTTIDESDMNLLPDLGTATLDPFRKAKTLNVKFFVHDPFTREAFSRDPRNVARKAEQYLASTGIADTCNFGAEAEFYLFDSVRYSTEMNSGFYEVDTEEGWWNRGKETNLDGTPNLGAKNRVKGGYFPVAPYDQTVDVRDDMVRNLAASGFALERFHHEVGGGQQEINYRFNTMLHAADDIQTFKYIIKNTARLHGKAATFMPKPLAGDNGSGMHAHQSLWKDGKPLFHDESGYAGLSDIARYYIGGILHHAGAVLAFTNATLNSYHRLVPGFEAPINLVYSQRNRSAAVRIPITGSNPKAKRIEFRAPDPSGNPYLGFAAMMMAGLDGIKNRIEPHAPVDKDVYELPPEEAASIPQAPTSLEASLKALQEDTDFLTESDVFTEDLIEAYIQYKYDNEISPVRLRPTPQEFELYFDC

SEQ ID NO: 7 - DNA, 22 bp, Artificial Sequence
  primer
gtggcgtttgaaaccccggaag

SEQ ID NO: 8 - DNA, 22 bp, Artificial Sequence
  primer
ttagcagtcgaagtacaattcg

SEQ ID NO: 9 - DNA, 40 bp, Artificial Sequence
  primer
ggggatcctctagagtcgaccttgattgatcatgtcgagg

SEQ ID NO: 10 - DNA, 42 bp, Artificial Sequence
  primer
ctatcggctagctaagtgaaggtgactcctcattgacatggg

SEQ ID NO: 11 - DNA, 42 bp, Artificial Sequence
  primer
cccatgtcaatgaggagtcaccttcacttagctagccgatag

SEQ ID NO: 12 - DNA, 40 bp, Artificial Sequence
  primer
gcttgcatgcctgcaggtcgactctggcgaggtccatatg

SEQ ID NO: 13 - DNA, 24 bp, Artificial Sequence
  primer
tgcaaggcgattaagttgggtaac

SEQ ID NO: 14 - DNA, 24 bp, Artificial Sequence
  primer
gaaacagctatgaccatgattacg

SEQ ID NO: 15 - DNA, 23 bp, Artificial Sequence
  primer
cgatgacatggttcgcaacctcg

SEQ ID NO: 16 - DNA, 20 bp, Artificial Sequence
  primer
gagcaaaccctcacatctca

SEQ ID NO: 17 - DNA, 46 bp, Artificial Sequence
  primer
gcatcgagccacacgctccagtgaacaaggacctctacgaactacc

SEQ ID NO: 18 - DNA, 46 bp, Artificial Sequence
  primer
ggtagttcgtagaggtccttgttcactggagcgtgtggctcgatgc

SEQ ID NO: 19 - DNA, 46 bp, Artificial Sequence
  primer
gcatcgagccacacgctccagtggaaaaggacctctacgaactacc

SEQ ID NO: 20 - DNA, 46 bp, Artificial Sequence
  primer
ggtagttcgtagaggtccttttccactggagcgtgtggctcgatgc

SEQ ID NO: 21 - DNA, 46 bp, Artificial Sequence
  primer
gcatcgagccacacgctccagtgcacaaggacctctacgaactacc

SEQ ID NO: 22 - DNA, 46 bp, Artificial Sequence
  primer
ggtagttcgtagaggtccttgtgcactggagcgtgtggctcgatgc

SEQ ID NO: 23 - DNA, 46 bp, Artificial Sequence
  primer
gcatcgagccacacgctccagtgagcaaggacctctacgaactacc

SEQ ID NO: 24 - DNA, 46 bp, Artificial Sequence
  primer
ggtagttcgtagaggtccttgctcactggagcgtgtggctcgatgc

SEQ ID NO: 25 - DNA, 46 bp, Artificial Sequence
  primer
gcatcgagccacacgctccagtggtcaaggacctctacgaactacc

SEQ ID NO: 26 - DNA, 46 bp, Artificial Sequence
  primer
ggtagttcgtagaggtccttgaccactggagcgtgtggctcgatgc

SEQ ID NO: 27 - DNA, 46 bp, Artificial Sequence
  primer
gcatcgagccacacgctccagtgaacaaggacctcttcgaactacc

SEQ ID NO: 28 - DNA, 46 bp, Artificial Sequence
  primer
ggtagttcgaagaggtccttgttcactggagcgtgtggctcgatgc

SEQ ID NO: 29 - DNA, 1434 bp, Artificial Sequence
  Corynebacterium glutamicum ATCC13032 Glutamine synthetase n.t
gtggcgtttgaaaccccggaagaaattgtcaagttcatcaaggatgaaaacgtcgagttcgttgacgttcgattcaccgaccttcccggcaccgagcagcacttcagcatcccagctgccagcttcgatgcagatacaatcgaagaaggtctcgcattcgacggatcctcgatccgtggcttcaccacgatcgacgaatctgacatgaatctcctgccagacctcggaacggccacccttgatccattccgcaaggcaaagaccctgaacgttaagttcttcgttcacgatcctttcacccgcgaggcattctcccgcgacccacgcaacgtggcacgcaaggcagagcagtacctggcatccaccggcattgcagacacctgcaacttcggcgccgaggctgagttctacctcttcgactccgttcgctactccaccgagatgaactccggcttctacgaagtagataccgaagaaggctggtggaaccgtggcaaggaaaccaacctcgacggcaccccaaacctgggcgcaaagaaccgcgtcaagggtggctacttcccagtagcaccatacgaccaaaccgttgacgtgcgcgatgacatggttcgcaacctcgcagcttccggcttcgctcttgagcgtttccaccacgaagtcggtggcggacagcaggaaatcaactaccgcttcaacaccatgctccacgcggcagatgatatccagaccttcaagtacatcatcaagaacaccgctcgcctccacggcaaggctgcaaccttcatgcctaagccactggctggcgacaacggttccggcatgcacgctcaccagtccctctggaaggacggcaagccactcttccacgatgagtccggctacgcaggcctgtccgacatcgcccgctactacatcggcggcatcctgcaccacgcaggcgctgttctggcgttcaccaacgcaaccctgaactcctaccaccgtctggttccaggcttcgaggctccaatcaacctggtgtactcacagcgcaaccgttccgctgctgtccgtatcccaatcaccggatccaacccgaaggcaaagcgcatcgaattccgcgctccagacccatcaggcaacccatacctgggctttgcagcgatgatgatggccggcctcgacggcatcaagaaccgcatcgagccacacgctccagtggacaaggacctctacgaactaccaccagaggaagctgcatccattccacaggcaccaacctccctggaagcatccctgaaggcactgcaggaagacaccgacttcctcaccgagtctgacgtcttcaccgaggatctcatcgaggcgtacatccagtacaagtacgacaacgagatctccccagttcgcctgcgcccaaccccgcaggaattcgaattgtacttcgactgctaa